European Patent Specification EP 3 973 053 B1, published January 18, 2023. Title: Mikroorganismen-Stamm und Verfahren zur fermentativen Herstellung von Gamma-Glutamyltyrosin und Gamma-Glutamylphenylalanin. Applicant: Wacker Chemie AG. The sequence listing filed with the application follows.

SEQUENCE LISTING (2 sequences)

SEQ ID NO: 1 - DNA, 1557 bp, Escherichia coli
atgatcccggacgtatcacaggcgctggcctggctggaaaaacatcctcaggcgttaaaggggatacagcgtgggctggagcgcgaaactttgcgtgttaatgctgatggcacactggcaacaacaggtcatcctgaagcattaggttccgcactgacgcacaaatggattactaccgattttgcggaagcattgctggaattcattacaccagtggatggtgatattgaacatatgctgacctttatgcgcgatctgcatcgttatacggcgcgcaatatgggcgatgagcggatgtggccgttaagtatgccatgctacatcgcagaaggtcaggacatcgaactggcacagtacggcacttctaacaccggacgctttaaaacgctgtatcgtgaagggctgaaaaatcgctacggcgcgctgatgcaaaccatttccggcgtgcactacaatttctctttgccaatggcattctggcaagcgaagtgcggtgatatctcgggcgctgatgccaaagagaaaatttctgcgggctatttccgcgttatccgcaattactatcgtttcggttgggtcattccttatctgtttggtgcatctccggcgatttgttcttctttcctgcaaggaaaaccaacgtcgctgccgtttgagaaaaccgagtgcggtatgtattacctgccgtatgcgacctctcttcgtttgagcgatctcggctataccaataaatcgcaaagcaatcttggtattaccttcaacgatctttacgagtacgtagcgggccttaaacaggcaatcaaaacgccatcggaagagtacgcgaagattggtattgagaaagacggtaagaggctgcaaatcaacagcaacgtgttgcagattgaaaacgaactgtacgcgccgattcgtccaaaacgcgttacccgcagcggcgagtcgccttctgatgcgctgttacgtggcggcattgaatatattgaagtgcgttcgctggacatcaacccgttctcgccgattggtgtagatgaacagcaggtgcgattcctcgacctgtttatggtctggtgtgcgctggctgatgcaccggaaatgagcagtagcgaacttgcctgtacacgcgttaactggaaccgggtgatcctcgaaggtcgcaaaccgggtctgacgctgggtatcggctgcgaaaccgcacagttcccgttaccgcaggtgggtaaagatctgttccgcgatctgaaacgcgtcgcgcaaacgctggatagtattaacggcggcgaagcgtatcagaaagtgtgtgatgaactggttgcctgcttcgataatcccgatctgactttctctgcccgtatcttaaggtctatgattgatactggtattggcggaacaggcaaagcatttgcagaagcctaccgtaatctgctgcgtgaagagccgctggaaattctgcgcgaagaggattttgtagccgagcgcgaggcgtctgaacgccgtcagcaggaaatggaagccgctgataccgaaccgtttgcggtgtggctggaaaaacacgcctga

SEQ ID NO: 2 - protein, 518 aa, Escherichia coli
MIPDVSQALAWLEKHPQALKGIQRGLERETLRVNADGTLATTGHPEALGSALTHKWITTDFAEALLEFITPVDGDIEHMLTFMRDLHRYTARNMGDERMWPLSMPCYIAEGQDIELAQYGTSNTGRFKTLYREGLKNRYGALMQTISGVHYNFSLPMAFWQAKCGDISGADAKEKISAGYFRVIRNYYRFGWVIPYLFGASPAICSSFLQGKPTSLPFEKTECGMYYLPYATSLRLSDLGYTNKSQSNLGITFNDLYEYVAGLKQAIKTPSEEYAKIGIEKDGKRLQINSNVLQIENELYAPIRPKRVTRSGESPSDALLRGGIEYIEVRSLDINPFSPIGVDEQQVRFLDLFMVWCALADAPEMSSSELACTRVNWNRVILEGRKPGLTLGIGCETAQFPLPQVGKDLFRDLKRVAQTLDSINGGEAYQKVCDELVACFDNPDLTFSARILRSMIDTGIGGTGKAFAEAYRNLLREEPLEILREEDFVAEREASERRQQEMEAADTEPFAVWLEKHA